European Patent Application EP 4 435 010 A1, published September 25, 2024. Title: Bispecific Antibody against TIGIT and PD-L1, and Pharmaceutical Composition Thereof and Use Thereof. Applicant: BIOTHEUS INC. The sequence listing filed with the application follows.

SEQUENCE LISTING (23 sequences)

SEQ ID NO: 1 - protein, 451 aa, synthetic construct
  source 1..451: note = Anti-TIGIT intact wild-type IgG1 antibody heavy chain
QLQLQESGPGLVKPAETLSLTCTVSGGSISSYDHYWTWIRQPPGKGLEWIGTVYYSGSTFHNPSLKSRVTIPVDTSKNQFSLKLSSVTAADTAVYYCARVGPDVSHPPFDYWGQGTLVTVSSASTKGPSVFPLAPSSKSTSGGTAALGCLVKDYFPEPVTVSWNSGALTSGVHTFPAVLQSSGLYSLSSVVTVPSSSLGTQTYICNVNHKPSNTKVDKKVEPKSCDKTHTCPPCPAPELLGGPSVFLFPPKPKDTLMISRTPEVTCVVVDVSHEDPEVKFNWYVDGVEVHNAKTKPREEQYNSTYRVVSVLTVLHQDWLNGKEYKCKVSNKALPAPIEKTISKAKGQPREPQVYTLPPSRDELTKNQVSLTCLVKGFYPSDIAVEWESNGQPENNYKTTPPVLDSDGSFFLYSKLTVDKSRWQQGNVFSCSVMHEALHNHYTQKSLSLSPG

SEQ ID NO: 2 - protein, 10 aa, synthetic construct
  source 1..10: note = Linker G4S
GGGGSGGGGS

SEQ ID NO: 3 - protein, 115 aa, synthetic construct
  source 1..115: note = Anti-PD-L1 single-domain antibody (VHH)
EVQLQESGGGLVQPGGSLRLSCAASGFTFSSYWMYWLRQAPGKGLEWVSSINSDSSSTYYRDSVKGRFTISRDNAKNTLYLQMNSLKSEDTAVYYCAKDPGGYAKGQGTQVTVSS

SEQ ID NO: 4 - protein, 576 aa, synthetic construct
  source 1..576: note = Anti-TIGIT/anti-PD-L1 bispecific antibody peptide chain #1
QLQLQESGPGLVKPAETLSLTCTVSGGSISSYDHYWTWIRQPPGKGLEWIGTVYYSGSTFHNPSLKSRVTIPVDTSKNQFSLKLSSVTAADTAVYYCARVGPDVSHPPFDYWGQGTLVTVSSASTKGPSVFPLAPSSKSTSGGTAALGCLVKDYFPEPVTVSWNSGALTSGVHTFPAVLQSSGLYSLSSVVTVPSSSLGTQTYICNVNHKPSNTKVDKKVEPKSCDKTHTCPPCPAPELLGGPSVFLFPPKPKDTLMISRTPEVTCVVVDVSHEDPEVKFNWYVDGVEVHNAKTKPREEQYNSTYRVVSVLTVLHQDWLNGKEYKCKVSNKALPAPIEKTISKAKGQPREPQVYTLPPSRDELTKNQVSLTCLVKGFYPSDIAVEWESNGQPENNYKTTPPVLDSDGSFFLYSKLTVDKSRWQQGNVFSCSVMHEALHNHYTQKSLSLSPGGGGGSGGGGSEVQLQESGGGLVQPGGSLRLSCAASGFTFSSYWMYWLRQAPGKGLEWVSSINSDSSSTYYRDSVKGRFTISRDNAKNTLYLQMNSLKSEDTAVYYCAKDPGGYAKGQGTQVTVSS

SEQ ID NO: 5 - protein, 214 aa, synthetic construct
  source 1..214: note = Anti-TIGIT/anti-PD-L1 bispecific antibody peptide chain #2 (anti-TIGIT kappa light chain)
DIQMTQSPSSLSASVGDRVTITCRASQSISSYLNWYQQKPGKAPKLLIYAASSLQSGVPSRFSGSGSGTDFTLTISSLQPEDFATYYCQQSYSTPITFGGGTKVEIKRTVAAPSVFIFPPSDEQLKSGTASVVCLLNNFYPREAKVQWKVDNALQSGNSQESVTEQDSKDSTYSLSSTLTLSKADYEKHKVYACEVTHQGLSSPVTKSFNRGEC

SEQ ID NO: 6 - protein, 220 aa, synthetic construct
  source 1..220: note = Human PD-L1 extracellular fragment amino acid sequence
FTVTVPKDLYVVEYGSNMTIECKFPVEKQLDLAALIVYWEMEDKNIIQFVHGEEDLKVQHSSYRQRARLLKDQLSLGNAALQITDVKLQDAGVYRCMISYGGADYKRITVKVNAPYNKINQRILVVDPVTSEHELTCQAEGYPKAEVIWTSSDHQVLSGKTTTTNSKREEKLFNVTSTLRINTTTNEIFYCTFRRLDPEENHTAELVIPELPLAHPPNER

SEQ ID NO: 7 - protein, 221 aa, synthetic construct
  source 1..221: note = Cynomolgus monkey PD-L1 extracellular fragment amino acid sequence
FTVTVPKDLYVVEYGSNMTIECKFPVEKQLDLTSLIVYWEMEDKNIIQFVHGEEDLKVQHSNYRQRAQLLKDQLSLGNAALRITDVKLQDAGVYRCMISYGGADYKRITVKVNAPYNKINQRILVVDPVTSEHELTCQAEGYPKAEVIWTSSDHQVLSGKTTTTNSKREEKLLNVTSTLRINTTANEIFYCIFRRLDPEENHTAELVIPELPLALPPNERT

SEQ ID NO: 8 - protein, 120 aa, synthetic construct
  source 1..120: note = Human TIGIT extracellular fragment amino acid sequence
MMTGTIETTGNISAEKGGSIILQCHLSSTTAQVTQVNWEQQDQLLAICNADLGWHISPSFKDRVAPGPGLGLTLQSLTVNDTGEYFCIYHTYPDGTYTGRIFLEVLESSVAEHGARFQIP

SEQ ID NO: 9 - protein, 120 aa, synthetic construct
  source 1..120: note = Cynomolgus monkey TIGIT extracellular fragment amino acid sequence
MMTGTIETTGNISAKKGGSVILQCHLSSTMAQVTQVNWEQHDHSLLAIRNAELGWHIYPAFKDRVAPGPGLGLTLQSLTMNDTGEYFCTYHTYPDGTYRGRIFLEVLESSVAEHSARFQI

SEQ ID NO: 10 - protein, 7 aa, synthetic construct
  source 1..7: note = HCDR1 of anti-TIGIT intact wild-type IgG1 heavy chain antibody
SYDHYWT

SEQ ID NO: 11 - protein, 16 aa, synthetic construct
  source 1..16: note = HCDR2 of anti-TIGIT intact wild-type IgG1 heavy chain antibody
TVYYSGSTFHNPSLKS

SEQ ID NO: 12 - protein, 12 aa, synthetic construct
  source 1..12: note = HCDR3 of anti-TIGIT intact wild-type IgG1 heavy chain antibody
VGPDVSHPPFDY

SEQ ID NO: 13 - protein, 11 aa, synthetic construct
  source 1..11: note = LCDR1 of anti-TIGIT kappa light chain
RASQSISSYLN

SEQ ID NO: 14 - protein, 7 aa, synthetic construct
  source 1..7: note = LCDR2 of anti-TIGIT kappa light chain
AASSLQS

SEQ ID NO: 15 - protein, 9 aa, synthetic construct
  source 1..9: note = LCDR3 of anti-TIGIT kappa light chain
QQSYSTPIT

SEQ ID NO: 16 - protein, 5 aa, synthetic construct
  source 1..5: note = HCDR1 of anti-PD-L1 VHH
SYWMY

SEQ ID NO: 17 - protein, 17 aa, synthetic construct
  source 1..17: note = HCDR2 of anti-PD-L1 VHH
SINSDSSSTYYRDSVKG

SEQ ID NO: 18 - protein, 6 aa, synthetic construct
  source 1..6: note = HCDR3 of anti-PD-L1 VHH
DPGGYA

SEQ ID NO: 19 - protein, 122 aa, synthetic construct
  source 1..122: note = Anti-TIGIT intact wild-type IgG1 heavy chain variable region (VH)
QLQLQESGPGLVKPAETLSLTCTVSGGSISSYDHYWTWIRQPPGKGLEWIGTVYYSGSTFHNPSLKSRVTIPVDTSKNQFSLKLSSVTAADTAVYYCARVGPDVSHPPFDYWGQGTLVTVSS

SEQ ID NO: 20 - protein, 107 aa, synthetic construct
  source 1..107: note = Anti-TIGIT kappa light chain variable region (VL)
DIQMTQSPSSLSASVGDRVTITCRASQSISSYLNWYQQKPGKAPKLLIYAASSLQSGVPSRFSGSGSGTDFTLTISSLQPEDFATYYCQQSYSTPITFGGGTKVEIK

SEQ ID NO: 21 - protein, 120 aa, synthetic construct
  source 1..120: note = Mouse TIGIT extracellular fragment amino acid sequence
TIDTKRNISAEEGGSVILQCHFSSDTAEVTQVDWKQQDQLLAIYSVDLGWHVASVFSDRVVPGPSLGLTFQSLTMNDTGEYFCTYHTYPGGIYKGRIFLKVQESSDDRNGLAQFQTAPLG

SEQ ID NO: 22 - protein, 5 aa, synthetic construct
  source 1..5: note = GGGGS in linker
GGGGS

SEQ ID NO: 23 - protein, 20 aa, synthetic construct
  source 1..20: note = linker
GGGGSGGGGSGGGGSGGGGS